European Patent Application EP 4 796 563 A1, published August 26, 2026. Title: 一种全人源TSH受体阻断性单克隆抗体及其制备和应用. Applicant: 上海交通大学医学院附属第九人民医院. Application CN. The sequence listing filed with the application follows.

SEQUENCE LISTING (11 sequences)

SEQ ID NO: 1 - protein, 124 aa, synthetic construct
VHSEVQLVESGGGLVQPGGSLRLSCVASGFDFNQYSMNWVRQAPGKGLEWLSYISSSAATVFYADSVQGRLTISRDNGKNSLFLQMNSLRVEDTAVYYCVREAVIVDGMPFEYWGQGALVTVSS

SEQ ID NO: 2 - protein, 110 aa, synthetic construct
VHSEIVLTQSPGTLSLSPGERATLSCRASQSVTSSQLAWYQQKPGQAPRLLIYGESSRATGIPDRFSGRGSGTDFALTISRLEPEDFAVYCCQQYGTSIAFGGGTKVEIK

SEQ ID NO: 3 - DNA, 374 bp, synthetic construct
  source 1..374: mol_type = other DNA
gtacattctgaggtgcagctggtggagtccggtggaggcttggttcaaccgggggggtccctgagactctcctgtgtagcctctggattcgacttcaaccaatatagcatgaactgggtccgccaggctccagggaagggactggagtggctttcatacatcagtagcagcgctgcaaccgtgttctacgcagactctgtgcagggccgactcaccatctccagagacaatggcaagaattcactctttctgcagatgaacagcctgagagtcgaggacacggctgtctattactgtgtcagagaagctgttatagtggatggcatgccgtttgaatactggggccagggagccctggtcaccgtctcctcagc

SEQ ID NO: 4 - DNA, 330 bp, synthetic construct
  source 1..330: mol_type = other DNA
gtacattcagaaattgtgttgacgcagtctccaggcaccctgtctttgtctccaggggaaagagccaccctctcctgcagggccagtcagagtgttaccagcagccagttagcctggtaccagcagaaacctggccaggctcccagactcctcatctatggtgaatccagcagggccactggcatcccagacaggttcagtggcagggggtctgggacagacttcgctctcaccatcagcagactggagcctgaagattttgcagtgtattgctgtcagcagtatggtacttcaatcgctttcggcggagggaccaaggtggagatcaaa

SEQ ID NO: 5 - protein, 764 aa, synthetic construct
MRPADLLQLVLLLDLPRDLGGMGCSSPPCECHQEEDFRVTCKDIQRIPSLPPSTQTLKLIETHLRTIPSHAFSNLPNISRIYVSIDVTLQQLESHSFYNLSKVTHIEIRNTRNLTYIDPDALKELPLLKFLGIFNTGLKMFPDLTKVYSTDIFFILEITDNPYMTSIPVNAFQGLCNETLTLKLYNNGFTSVQGYAFNGTKLDAVYLNKNKYLTVIDKDAFGGVYSGPSLLDVSQTSVTALPSKGLEHLKELIARNTWTLKKLPLSLSFLHLTRADLSYPSHCCAFKNQKKIRGILESLMCNESSMQSLRQRKSVNALNSPLHQEYEENLGDSIVGYKEKSKFQDTHNNAHYYVFFEEQEDEIIGFGQELKNPQEETLQAFDSHYDYTICGDSEDMVCTPKSDEFNPCEDIMGYKFLRIVVWFVSLLALLGNVFVLLILLTSHYKLNVPRFLMCNLAFADFCMGMYLLLIASVDLYTHSEYYNHAIDWQTGPGCNTAGFFTVFASELSVYTLTVITLERWYAITFAMRLDRKIRLRHACAIMVGGWVCCFLLALLPLVGISSYAKVSICLPMDTETPLALAYIVFVLTLNIVAFVIVCCCYVKIYITVRNPQYNPGDKDTKIAKRMAVLIFTDFICMAPISFYALSAILNKPLITVSNSKILLVLFYPLNSCANPFLYAIFTKAFQRDVFILLSKFGICKRQAQAYRGQRVPPKNSTDIQVQKVTHEMRQGLHNMEDVYELIENSHLTPKKQGQISEEYMQTVL

SEQ ID NO: 6 - protein, 5 aa, synthetic construct
QYSMN

SEQ ID NO: 7 - protein, 17 aa, synthetic construct
YISSSAATVFYADSVQG

SEQ ID NO: 8 - protein, 12 aa, synthetic construct
EAVIVDGMPFEY

SEQ ID NO: 9 - protein, 12 aa, synthetic construct
RASQSVTSSQLA

SEQ ID NO: 10 - protein, 7 aa, synthetic construct
GESSRAT

SEQ ID NO: 11 - protein, 8 aa, synthetic construct
QQYGTSIA